European Patent Application EP 4 786 598 A1, published August 5, 2026. Title: Polynucleotides encoding virus-derived proteins. Applicant: Shionogi and Co., Ltd. The sequence listing filed with the application follows.

SEQUENCE LISTING (218 sequences)

SEQ ID NO: 1 - RNA, 44 nt, synthetic construct
  source 1..44: mol_type = other RNA
aaataagagagaaaagaagagtaagaagaaatataagagccacc

SEQ ID NO: 2 - RNA, 54 nt, synthetic construct
  source 1..54: mol_type = other RNA
aaataagagagaaaagaagagtaagaagaaatataagaccccggcgccgccacc

SEQ ID NO: 3 - RNA, 61 nt, synthetic construct
  source 1..61: mol_type = other RNA
agacccaagctacatttgcttctgacacaactgtgttcactagcaacctcaaacagacacc

SEQ ID NO: 4 - RNA, 47 nt, synthetic construct
  source 1..47: mol_type = other RNA
gggaaataagagagaaaagaagagtaagaagaaatataagagccacc

SEQ ID NO: 5 - RNA, 57 nt, synthetic construct
  source 1..57: mol_type = other RNA
gggaaataagagagaaaagaagagtaagaagaaatataagaccccggcgccgccacc

SEQ ID NO: 6 - RNA, 64 nt, synthetic construct
  source 1..64: mol_type = other RNA
gggagacccaagctacatttgcttctgacacaactgtgttcactagcaacctcaaacagacacc

SEQ ID NO: 7 - RNA, 341 nt, synthetic construct
  source 1..341: mol_type = other RNA
ggtctctctagctagaccagatctgagcccgggagctctctggctaactagggaacccactgcttaagcctcaataaagcttgccttgagtgcttcaagtagtgtgtgcccgtctgttgtgtgactctggtaactagagatccctcagacccttttagtcagtgtggaaaatctctagcagtggcgcccgaacagggaccttaaagtgaaagtggaaccagaggagctctctcgacgcaggactcggcttgcttagcgcgcacggcaagaggcgaggggcggcgactgaattgggtgtcaacatagcagaataggcattactcgacagagaagagcaagaa

SEQ ID NO: 8 - RNA, 104 nt, synthetic construct
  source 1..104: mol_type = other RNA
agagcggccgctttttcagcaagattaagcccagggcagagccatctattgcttacatttgcttctgacacaactgtgttcactagcaacctcaaacagacacc

SEQ ID NO: 9 - RNA, 50 nt, synthetic construct
  source 1..50: mol_type = other RNA
ataaactagtattcttctggtccccacagactcagagagaacccgccacc

SEQ ID NO: 10 - RNA, 37 nt, synthetic construct
  source 1..37: mol_type = other RNA
actcttctggtccccacagactcagagagaacccacc

SEQ ID NO: 11 - RNA, 37 nt, synthetic construct
  source 1..37: mol_type = other RNA
actcttctggtccccacagactcagagagaagccacc

SEQ ID NO: 12 - RNA, 40 nt, synthetic construct
  source 1..40: mol_type = other RNA
actcttctggtccccacagactcagagagaacccgccacc

SEQ ID NO: 13 - RNA, 75 nt, synthetic construct
  source 1..75: mol_type = other RNA
aggatgtcttctggcaatttcatataagtattttttcaaaaatgtctcttctgtcaaccccacgcctttggcaca

SEQ ID NO: 14 - RNA, 12 nt, synthetic construct
  source 1..12: mol_type = other RNA
agaaagcttacc

SEQ ID NO: 15 - RNA, 73 nt, synthetic construct
  source 1..73: mol_type = other RNA
cagggcagagccatctattgcttacatttgcttctgacacaactgtgttcactagcaacctcaaacagacacc

SEQ ID NO: 16 - RNA, 71 nt, synthetic construct
  source 1..71: mol_type = other RNA
tcccgcagtcggcgtccagcggctctgcttgttcgtgtgtgtgtcgttgcaggccttattcaagcttgagg

SEQ ID NO: 17 - RNA, 44 nt, synthetic construct
  source 1..44: mol_type = other RNA
atgggcggcgcatgagagaagcccagaccaattacctacccaaa

SEQ ID NO: 18 - RNA, 15 nt, synthetic construct
  source 1..15: mol_type = other RNA
aggagaaagcttacc

SEQ ID NO: 19 - RNA, 44 nt, synthetic construct; identical to SEQ ID NO: 17
  source 1..44: mol_type = other RNA

SEQ ID NO: 20 - RNA, 84 nt, synthetic construct
  source 1..84: mol_type = other RNA
gggtctgcgtctataaaagagtgaggcgtcggcgccggagtaccgtttcctggttgtggccgttcgtctgtttgcgctttcgtg

SEQ ID NO: 21 - RNA, 111 nt, synthetic construct
  source 1..111: mol_type = other RNA
ccagccctccgtcacctcttcaccgcaccctcggactgccccaaggcccccgccgccgctccagcgccgcgcagccaccgccgccgccgccgcctctccttagtcgccgcc

SEQ ID NO: 22 - RNA, 283 nt, synthetic construct
  source 1..283: mol_type = other RNA
agagcgtcgggatatcgggtggcggctcgggacggaggacgcgctagtgtgagtgcgggcttctagaactacaccgaccctcgtgtcctcccttcatcctgcggggctggctggagcggccgctccggtgctgtccagcagccatagggagccgcacggggagcgggaaagcggtcgcggccccaggcggggcggccgggatggagcggggccgcgagcctgtggggaaggggctgtggcggcgcctcgagcggctgcaggttcttctgtgtggcagttcaga

SEQ ID NO: 23 - RNA, 24 nt, synthetic construct
  source 1..24: mol_type = other RNA
agagcttactctggctttgccgag

SEQ ID NO: 24 - RNA, 147 nt, synthetic construct
  source 1..147: mol_type = other RNA
aggaagattgtgcatgccgtgggtctgacggcttgagtagcgctagggagaatccctgcaggtaatatttgacttttgcttcatattaatctgagtggaaaataaaagggccctcttctcctctcgcttccctgccgggcaggcgcc

SEQ ID NO: 25 - RNA, 32 nt, synthetic construct
  source 1..32: mol_type = other RNA
gcacaagggaactgactcaggaggcagagaag

SEQ ID NO: 26 - RNA, 150 nt, synthetic construct
  source 1..150: mol_type = other RNA
gtcagtttcctcggcagcggtaggcgagagcacgcggaggagcgtgcgcgggggccccgggagacggcggcggtggcggcgcgggcagagcaaggacgcggcggatcccactcgcacagcagcgcactcggtgccccgcgcagggtcgcg

SEQ ID NO: 27 - RNA, 263 nt, synthetic construct
  source 1..263: mol_type = other RNA
ttagttggcgcgtagctttaccacaaaattcctggaattgccgtacgcttcgcagttgtttcaagttgtctaagggacatacgattttttttgcctctgcgtcacgattttaacccaaaagcgagtttagttacatgtacattattattagataaagaagtatcgcgaatacttcagttgaataaactgtgcttggtttttgggtgaggatttgtggaaagtagagtgcgcgataaccgtaactttcgacccggattttcgcc

SEQ ID NO: 28 - RNA, 27 nt, synthetic construct
  source 1..27: mol_type = other RNA
acaaggcgtgcaacgaccctgggcaag

SEQ ID NO: 29 - RNA, 148 nt, synthetic construct
  source 1..148: mol_type = other RNA
cacgacggagtgctcctataaaggcgcgggtcggtaccagacggcgtgaggagcgggagaggaagaggcctccggttgcaggtaagtgcaacacaaaaaagaaatagctgtcttttatccaggaaggggtaataagatagagtgggag

SEQ ID NO: 30 - RNA, 35 nt, synthetic construct
  source 1..35: mol_type = other RNA
agtacacagagagaaaggctaaagttctctggagg

SEQ ID NO: 31 - RNA, 51 nt, synthetic construct
  source 1..51: mol_type = other RNA
cttcttcctcggcgctgcctacgaggtggctgccatctgttttacggcatc

SEQ ID NO: 32 - RNA, 170 nt, synthetic construct
  source 1..170: mol_type = other RNA
gaattcgggcatccagacagtgggccgccggtctcagcaactagctcgctaggcagagggaggccaagagagtcgcagacggagtctcgagaccgaagccgaagcgggatccacagagcgcagcctgcccgcgcacccggtgccgcgaaagcctccagcgcagcgcggcc

SEQ ID NO: 33 - RNA, 167 nt, synthetic construct
  source 1..167: mol_type = other RNA
agcagaagctccctcagcgaggacagcaagggactagccaggagggagaacagaaactccagaacatcttggaaatagctcccagaaaagcaagcagccaaccaggcaggttctgtccctttcactcactggcccaaggcgccacatctccctccagaaaagacacc

SEQ ID NO: 34 - RNA, 431 nt, synthetic construct
  source 1..431: mol_type = other RNA
gggaggcccacgtatggcgcctctccaaaggctgcagaagtttcttgctaacaaaaagtccgcacattcgagcaaagacaggctttagcgagttattaaaaacttaggggcgctcttgtcccccacagggcccgaccgcacacagcaaggcgatggcccagctgtaagttggtagcactgagaactagcagcgcgcgcggagcccgctgagacttgaatcaatctggtctaacggtttcccctaaaccgctaggagccctcaatcggcgggacagcagggcgcgtcctctgccactctcgctccgaggtccccgcgccagagacgcagccgcgctcccaccacccacacccaccgcgccctcgttcgcctcttctccgggagccagtccgcgccaccgccgccgcccaggccatcgccaccctccgcagcc

SEQ ID NO: 35 - RNA, 532 nt, synthetic construct
  source 1..532: mol_type = other RNA
ggcaccccattcctggcctctgtctcccgcaccctatcccttcacagcctgtgctctaggggactggagatttccaaaacctgacccgatccctccccagttcagttccttctactgctttgggtggaaggctggtcgttgtgttaaaaggcaggaagggagaaagttgcatttaaactttaggagctgcgtcacggcagtctcctggagaaagctccgccgaacgggacagattctttttgcaacttggaggcgccgggcgtggggaggaggcggcgcgtggggcgggggcgcgcggggccggggtgcaggcggggacgcggggtgacgcgggcccgggccgctgtagcacacaggggctcggtctctcggcttcaggcggagtccggctgcactaggctgggagcgcggcgggacgcgaaccgggaggctggcagcccgcgggcgagccgcgctggggggccgaggccggggtcggggccggggagccccgagagctgccgcagcggggtcccggggccgcggaggggcc

SEQ ID NO: 36 - RNA, 473 nt, synthetic construct
  source 1..473: mol_type = other RNA
tagcatgttcgcactggcacactgcggtcacactggcttcgctcagcaaaatattgcttgggtaatttttttttttagttgctaatttattgttttcaacgctgttgcacagtgtgcagcataaccattaacaatgacttgagacctctcaaacgtaaaccaattttttttttttttttgcacgtgaaacatagtgataacgaagccacaaaagtgaaaccaacaaaaagcgttccagtaaagttaccattagataatgaaatcgaggattaacgcggtctaagcatgtgtaactgagctcctacgggcgaggaattgcaggtaactagcccaggaggcaccaggtagcggagcaggtggcgtgggtcggaccgacaaggcacttacttggccagcggagtctcacttttgggctgaaaaacgtaaacaaacagcggcgtgcgtacagtcccgggcataaaaatatagccatc

SEQ ID NO: 37 - RNA, 587 nt, synthetic construct
  source 1..587: mol_type = other RNA
agaggcggagaagaagaggtagcgagtggacgtgactgctctatcccgggcaaaagggatagaaccagaggtggggagtctgggcagtcggcgacccgcgaagacttgaggtgccgcagcggcatccggagtagcgccgggctccctccggggtgcagccgccgtcgggggaagggcgccacaggccgggaagacctcctccctttgtgtccagtagtggggtccaccggagggcggcccgtgggccgggcctcaccgcggcgctccgggactgtggggtcaggctgcgttgggtggacgcccacctcgccaaccttcggaggtccctgggggtcttcgtgcgccccggggctgcagagatccaggggaggcgcctgtgaggcccggacctgccccggggcgaagggtatgtggcgagacagagccctgcacccctaattcccggtggaaaactcctgttgccgtttccctccaccggcctggagtctcccagtcttgtcccggcagtgccgccctccccactaagacctaggcgcaaaggcttggctcatggttgacagctcagagagagaaagatctgagggaag

SEQ ID NO: 38 - RNA, 363 nt, synthetic construct
  source 1..363: mol_type = other RNA
aactcgctgtagtaattccagcgagaggcagagggagcgagcgggcggccggctagggtggaagagccgggcgagcagagctgcgctgcgggcgtcctgggaagggagatccggagcgaatagggggcttcgcctctggcccagccctcccgctgatcccccagccagcggtccgcaacccttgccgcatccacgaaactttgcccatagcagcgggcgggcactttgcactggaacttacaacacccgagcaaggacgcgactctcccgacgcggggaggctattctgcccatttggggacacttccccgccgctgccaggacccgcttctctgaaaggctctccttgcagctgcttagacg

SEQ ID NO: 39 - RNA, 111 nt, synthetic construct
  source 1..111: mol_type = other RNA
atacaggaagtgacgatacttttggcgcgcgcggttgctgtttcttctctggctccgggaccggcggcggcggcggcggcacgggcggcggcgtagggtgttttaactcaa

SEQ ID NO: 40 - RNA, 155 nt, synthetic construct
  source 1..155: mol_type = other RNA
aaccgcatctgcagcgagcatctgagaagccaagactgagccggcggccgcggcgcagcgaacgagcagtgaccgtgctcctacccagctctgctccacagcgcccacctgtctccgcccctcggcccctcgcccggctttgcctaaccgccacg

SEQ ID NO: 41 - RNA, 341 nt, synthetic construct
  source 1..341: mol_type = other RNA
agctggattcagcgtgtccgcgacctcacctttaggtcctgtgaggtcggtggaatcctggggtcctccaaatctaccaggccatctccccagtttcccagttcttcctgcgtgcgggcgagagtggttgggccctcgggaacccactcagagcgaggctaaatttacggagggactttctgttagcagcatgagggcctgtggttagacctatagaggtatttcctttgatttaagccagaaagtcctgagagcggatcggggagcatttgcggatcggtcactttttcctcctttctgagtctcttatcccctaccacagggacggcccaggtggcagg

SEQ ID NO: 42 - RNA, 20 nt, synthetic construct
  source 1..20: mol_type = other RNA
ggatcactttcctccaagcg

SEQ ID NO: 43 - RNA, 128 nt, synthetic construct
  source 1..128: mol_type = other RNA
catgcattattgtctcagtgcagttgtcagttgcagttcagcagacgggctaacgagtacttgcatctcttcaaatttacttaattgatcaaatcgaaagagcctgctaaagcaaaaaagaagtcacc

SEQ ID NO: 44 - RNA, 63 nt, synthetic construct
  source 1..63: mol_type = other RNA
agaacagagccagcgctgaagcaaggagcatcgtcacacaataacgttatactatctcttaaa

SEQ ID NO: 45 - RNA, 72 nt, synthetic construct
  source 1..72: mol_type = other RNA
acatcacattcaatcgcaacgttgaacagccaagatcagtcgaccaagcaagcaaactactaactagcaaaa

SEQ ID NO: 46 - RNA, 15 nt, synthetic construct
  source 1..15: mol_type = other RNA
gcatttctccccgag

SEQ ID NO: 47 - RNA, 57 nt, synthetic construct
  source 1..57: mol_type = other RNA
aaccctaagtgaccagctacaatcatagaccatcagcaagcaggtcattgttccaac

SEQ ID NO: 48 - RNA, 68 nt, synthetic construct
  source 1..68: mol_type = other RNA
ggaacaacnnggccgcctcgcgccgcccgccccggctctgactgaccgcgttactcccacagccagcc

SEQ ID NO: 49 - RNA, 216 nt, synthetic construct
  source 1..216: mol_type = other RNA
ctgatcgctgtagaccttacagttgctgctaactgccctggtgtgtgtgagggagagagagggagagagagggagagggagggagggagggagggagagcgcgctagcgcgagagagcgagtgagcaagcgagcagaaaagaggtggagagggggggaataaggaagagaggaggaaaggagagaaggcaggaagaaggcaggggaagataccacc

SEQ ID NO: 50 - RNA, 148 nt, synthetic construct
  source 1..148: mol_type = other RNA
agaagccccgggctcgtcagtcaaaccggttctctgtttgcactcggcagcacgggcaggcaagtggtccctaggttcgggagcagagcagcagcgcctcagtcctggtcccccagtcccaagcctcacctgcctgcccagcgccagg

SEQ ID NO: 51 - RNA, 37 nt, synthetic construct; identical to SEQ ID NO: 10
  source 1..37: mol_type = other RNA

SEQ ID NO: 52 - RNA, 594 nt, synthetic construct
  source 1..594: mol_type = other RNA
ggctaggtgtcccaccccgccttgtaagacaccggaaattcgtcaacgagcgatccctccgcgctccggaaccagaccgcggctggtcgtcaacctataaagtagtgcacttttctctcatggggcctttaggacgatctctaacgccacagttaccccccgagcacagcggagaagggttggggcgggcgagggcgtcagtgagaggcggtttggtggcgctgcggtaggatcacgtgaccacagtgggaggatacgcggtgtgctgcgtccctggccgaggctataaagggcgggtttagggcgtgccgccgccatttctgcttgctgtctgccggtttaagttgtgtgctcgggtgtccctttcctcttcccctcccgcagggcttgcggccaccatggcgtattagaggcagcagtgcctgcggcagcgttggcctttgcagcggcggcagcagcaccaggctctgcagcggcaacccccaccggcctaagccatggcgctcttcacgaaatccagcagcagtgttgctgtaacggacaaagataccttcgagttaagcacattcctcgaatccagcaaagccccacaac

SEQ ID NO: 53 - RNA, 37 nt, synthetic construct
  source 1..37: mol_type = other RNA
acttcatttcttctcaggctccaagaaggggaaaaaa

SEQ ID NO: 54 - RNA, 117 nt, synthetic construct
  source 1..117: mol_type = other RNA
ctgcagtgagattgaggggaaggcgcacgccggctatttatacatgtgagcgcgtcggtccctcccccagtagcgtcgcattttaccggcgcatccgtttcagcgagtcacacagca

SEQ ID NO: 55 - RNA, 25 nt, synthetic construct
  source 1..25: mol_type = other RNA
gggagagaaacaggttgttgggagt

SEQ ID NO: 56 - RNA, 297 nt, synthetic construct
  source 1..297: mol_type = other RNA
gtcccccgccctcccagtggcgcgcgtttacctgctttcaagcactgggaggcggggcgggagcggggtgcgcgcccgtccccggagcagccgctgtcagtcaccgccgctgcgcgccagggaggaccagcctctggctcaggcggcctgagcttcacgaccccggaacatagtatccgcgccccagcgacccctagcccagcgttgggtcccatccgccgggatcccgggatcctgggcccctcttggcctccgagcagcagccagcaccactcttgaacaccccattgggtcgcc

SEQ ID NO: 57 - RNA, 92 nt, synthetic construct
  source 1..92: mol_type = other RNA
acagcccacaaaattccacctgctcacaggttggctggctcgacccaggtggtgtcccctgctctgagccagctcccggccaagccagcacc

SEQ ID NO: 58 - RNA, 52 nt, synthetic construct
  source 1..52: mol_type = other RNA
agaacctacagccccacccagacccttggctgagccttctgcccagagcccc

SEQ ID NO: 59 - RNA, 44 nt, synthetic construct
  source 1..44: mol_type = other RNA
agaacctcagtggatctcagagagagccccagactgagggaagc

SEQ ID NO: 60 - RNA, 127 nt, synthetic construct
  source 1..127: mol_type = other RNA
atatataaaagtcacattgaagggtctacagctcaatttatcagccttctcaggtttactcaactttgagaaagcatcagctgctaatacatttgaaagaagattgtatcctaagacgtgtgttaat

SEQ ID NO: 61 - RNA, 118 nt, synthetic construct
  source 1..118: mol_type = other RNA
ctgcatatgaaactcaggcttgaagaactgcagtccagttcatcagctgtctggcttactccagcttaatacagggtcactcctgaaggatcctctctgagagtcattgtatgtgaag

SEQ ID NO: 62 - RNA, 128 nt, synthetic construct
  source 1..128: mol_type = other RNA
attcccaccgggacctgcggggctgagtgcccttctcggttgctgccgctgaggagcccgcccagccagccagggccgcgaggccgaggccaggccgcagcccaggagccgccccaccgcagctggcg

SEQ ID NO: 63 - RNA, 147 nt, synthetic construct
  source 1..147: mol_type = other RNA
cgattcaggaggttcgttccttttttaaaggaccctaatcactctgagtaccactgactcactcagtgtgcgcgattcatttcaaaaacgagccagcctcttcttccttcgtctactagatcagatccaaagcttcctcttccagct

SEQ ID NO: 64 - RNA, 116 nt, synthetic construct
  source 1..116: mol_type = other RNA
tgataataggctggagcctcggtggccatgcttcttgccccttgggcctccccccagcccctcctccccttcctgcacccgtacccccgtggtctttgaataaagtctgagctagc

SEQ ID NO: 65 - RNA, 122 nt, synthetic construct
  source 1..122: mol_type = other RNA
taataggctggagcctcggtggcctagcttcttgccccttgggcctccccccagcccctcctccccttcctgcacccgtacccccgtggtctttgaataaagtctgagtgggcggcgctagc

SEQ ID NO: 66 - RNA, 138 nt, synthetic construct
  source 1..138: mol_type = other RNA
gctcgctttcttgctgtccaatttctattaaaggttcctttgttccctaagtccaactactaaactgggggatattatgaagggccttgagcatctggattctgcctaataaaaaacatttattttcattgcgctagc

SEQ ID NO: 67 - RNA, 110 nt, synthetic construct
  source 1..110: mol_type = other RNA
tgataataggctggagcctcggtggccatgcttcttgccccttgggcctccccccagcccctcctccccttcctgcacccgtacccccgtggtctttgaataaagtctga

SEQ ID NO: 68 - RNA, 116 nt, synthetic construct
  source 1..116: mol_type = other RNA
taataggctggagcctcggtggcctagcttcttgccccttgggcctccccccagcccctcctccccttcctgcacccgtacccccgtggtctttgaataaagtctgagtgggcggc

SEQ ID NO: 69 - RNA, 132 nt, synthetic construct
  source 1..132: mol_type = other RNA
gctcgctttcttgctgtccaatttctattaaaggttcctttgttccctaagtccaactactaaactgggggatattatgaagggccttgagcatctggattctgcctaataaaaaacatttattttcattgc

SEQ ID NO: 70 - RNA, 122 nt, synthetic construct
  source 1..122: mol_type = other RNA
taataggctggagcctcggtggccatgcttcttgccccttgggcctccccccagcccctcctccccttcctgcacccgtacccccgtggtctttgaataaagtctgagtgggcggcgctagc

SEQ ID NO: 71 - RNA, 113 nt, synthetic construct
  source 1..113: mol_type = other RNA
taataggctggagcctcggtggccatgcttcttgccccttgggcctccccccagcccctcctccccttcctgcacccgtacccccgtggtctttgaataaagtctgagctagc

SEQ ID NO: 72 - RNA, 1073 nt, synthetic construct
  source 1..1073: mol_type = other RNA
tggatggattcttagcacttatctgggacgatctgcggagcctgtgcctcttcagctaccaccgcttgagagacttaatcttgattgtagcgaggattgtggaacttctgggacgcagggggtgggaagtcctgaaatattggtggaatctcctgcagtattggagccaggaactaaagaatagtgtcattagcttgctcaacgccacagctatagcagtagctgaggggacagatagggttatagaaatagtacaaagagcttatagagcttttctcaatatacctagaagaataagacagggcttggaaagggctttgctataagatgggtggcaagtggtcaaaatgtagtatgaagggatggcctactataagggaaagaatgaagcgagctgagctacagccacctgagccagcagcagaaggggtgggagcagcatctcgagacctggaaaaacatggagcaatcactagtagcaatacagcagctactaatgctgattgtgcctggctagaagcacaagaggatgaagaggtgggttttccagtcagacctcaggtacctttaagaccaatgacttacaagggagctttagatcttagccactttttaaaagaaaaggggggactggaagggctaatttactcccagaaaagacaagatattcttgatctgtgggtctatcacacacaaggctatttccctgattggcagaactacacaccagggccagggatcagatatccactgtgctttggatggtgcttcaagttagtaccaatggatccagaccaggtagaagaggccaacgaaggagagaacaacagcttgttacatcctataagcctgcatgggatggatgacccagagaaagaagtgttagtgtggaagtttgacagccgcctagcatttcgtcacatggcccgagaggtgcatccggagtactacaaagactgctgatgataataggctggagcctcggtggccatgcttcttgccccttgggcctccccccagcccctcctccccttcctgcacccgtacccccgtggtctttgaataaagtctga

SEQ ID NO: 73 - RNA, 81 nt, synthetic construct
  source 1..81: mol_type = other RNA
ccgggaagctcgacgcccggaagatccgcgagatcctgatcaaggccaagaagggcggcaagatcgccgtgtaagactagt

SEQ ID NO: 74 - RNA, 110 nt, synthetic construct
  source 1..110: mol_type = other RNA
gctggagcctcggtggccatgcttcttgccccttgggcctccccccagcccctcctccccttcctgcacccgtacccccgtggtctttgaataaagtctgagtgggcggc

SEQ ID NO: 75 - RNA, 110 nt, synthetic construct
  source 1..110: mol_type = other RNA
gctggagcctcggtagccgttcctcctgcccgctgggcctcccaacgggccctcctcccctccttgcaccggcccttcctggtctttgaataaagtctgagtgggcagca

SEQ ID NO: 76 - RNA, 29 nt, synthetic construct
  source 1..29: mol_type = other RNA
tgataataggctggagcctcggtggccat

SEQ ID NO: 77 - RNA, 266 nt, synthetic construct
  source 1..266: mol_type = other RNA
agctcgctttcttgctgtccaatttctattaaaggttcctttgttccctaagtccaactactaaactgggggatattatgaagggccttgagcatctggattctgcctaataaaaaacatttattttcattgcagctcgctttcttgctgtccaatttctattaaaggttcctttgttccctaagtccaactactaaactgggggatattatgaagggccttgagcatctggattctgcctaataaaaaacatttattttcattgc

SEQ ID NO: 78 - RNA, 110 nt, synthetic construct; identical to SEQ ID NO: 67
  source 1..110: mol_type = other RNA

SEQ ID NO: 79 - RNA, 79 nt, synthetic construct
  source 1..79: mol_type = other RNA
ggccactgctcgcgtcggcccgcgtctctgtgatataacccccgcgagctcctaaaaaggctcttttcagagccaccca

SEQ ID NO: 80 - RNA, 169 nt, synthetic construct
  source 1..169: mol_type = other RNA
gcctcgggctaatttccccatagccgtggggtgacttccctggtcaccaaggcagtgcatgcatgttggggtttcctttaccttttctataagttgtaccaaaacatccacttaagttctttgatttgtaccattccttcaaataaagaaatttggtacccaggtgttg

SEQ ID NO: 81 - RNA, 79 nt, synthetic construct; identical to SEQ ID NO: 79
  source 1..79: mol_type = other RNA

SEQ ID NO: 82 - RNA, 141 nt, synthetic construct
  source 1..141: mol_type = other RNA
gcctcgggctaatttccccatagccgtggggtgacttccctggtcaccaaggcagtgcatgcatgttggggtttcctttaccttttctataagttgtaccaaaacatccacttaagttctttgatttgtaccattccttca

SEQ ID NO: 83 - RNA, 71 nt, synthetic construct
  source 1..71: mol_type = other RNA
tacatatttgtttatgatggccacagcctaaagtacacacggctgtgacttgattcaaaagaaaatgttat

SEQ ID NO: 84 - RNA, 84 nt, synthetic construct
  source 1..84: mol_type = other RNA
atctgacttggtctctgttaatgacgtctctccctctaaaccccattaaggactgggagaggcagagcaagcctcagagcccag

SEQ ID NO: 85 - RNA, 79 nt, synthetic construct
  source 1..79: mol_type = other RNA
gagttgaccagtgtgcggatgataactactgacgaaagagtcatcgactcagttagtggttggatgtagtcacattagt

SEQ ID NO: 86 - RNA, 235 nt, synthetic construct
  source 1..235: mol_type = other RNA
aatgtctgtttcctttttcagaatttggttccaaaatttcatttcttactcattttcgtttctattatttgtacaatttccatttcattatttaatttcttatctactcatatctactcatatttaatttcttatctactcatatctaatcgtccactcgacctcaacttgtaatctttacgaattttgttttcttgttaataaacgtaataagtttaaaacatttattataaat

SEQ ID NO: 87 - RNA, 318 nt, synthetic construct
  source 1..318: mol_type = other RNA
gaccggccagatgaggctggccaagccggggagctgctctctcatgaaacaagagctagaaactcaggatggtcatcttggagggaccaaggggtgggccacagccatggtgggagtggcctggacctgccctgggccacactgaccctgatacaggcatggcagaagaatgggaatattttatactgacagaaatcagtaatatttatatatttatatttttaaaatatttatttatttatttatttaagttcatattccatatttattcaagatgttttaccgtaataattattattaaaaatatgcttctacttg

SEQ ID NO: 88 - RNA, 45 nt, synthetic construct
  source 1..45: mol_type = other RNA
atggcttgtgtgcatgttttatgtttaaataaaatcacaaaacct

SEQ ID NO: 89 - RNA, 884 nt, synthetic construct
  source 1..884: mol_type = other RNA
ggtgtcccacaccaccagcccggtctgctcccagtggcccaaggatctctcagagcacaggcagctggatgagactctcaaactgatagatctcagcagagccgggcctggggctctttccttcagccagcagtgatgtccagaagaatattcaggacactaacggctccaggattttaacaaaagactgttgctcagatctattcagacaagcaataggttttataattttttattactgattttgttattatttttttatcagccagagtctccttcacccacatccctggcttcaccctaaatggctcagtgcctgagggtggggaccaagccctgcctagacacttgccttctttgccaagctaatctgtagggccggacctatgacctaaggacacactaatcgaactgcaaactatgagtcttctaccccaagaggtggctatggccaccccttctatgggcctgggtctcccaaacctaggggtcaggctccattaggttttgcctattcccgtctcttcctatccaaccactcaaattaacctttccttgcctgagaccagttgggagcactggagtgcagggaggagaggggaagggccatactgggctgccaggtgctagtctcctttgtactgagggccagatgatcaccatgagaggaggagggccatgggaaaccgagaactcactattcaagaagacctggacactcctgccctgctgtgtatagttggaagatatttatatatattttttggttgtcaatattaaatacagacactaagttatagtatatctggacaaaccaacttgtaaatataccaccttactccctctgtaacttacctaagcagatataaatggctggtttttag

SEQ ID NO: 90 - RNA, 301 nt, synthetic construct
  source 1..301: mol_type = other RNA
aaattgcacacactcagtgcagcaatatattaccagcaagaataaaaaagaaatccatatcttaaagaaacagctttcaagtgcctttctgcagtttttcaggagcgcaagatagatttggaataggaataagctctagttcttaacaaccgacactcctacaagatttagaaaaaagtttacaacataatctagtttacagaaaaatcttgtgctagaatactttttaaaaggtattttgaataccattaaaactgcttttttttttccagcaagtatccaaccaacttggttctgcttc

SEQ ID NO: 91 - RNA, 19 nt, synthetic construct
  source 1..19: mol_type = other RNA
ctctctttagacactgtca

SEQ ID NO: 92 - RNA, 1048 nt, synthetic construct
  source 1..1048: mol_type = other RNA
gcaagacgactcatccctatatgtttgtttttttatgtgctcagtgatgtccaggtatcaatcctttaatagataatttttatgtacgttatggatggtcgaattcagcactgaattgcatccataacgtggtatcgtctttgatcctcttatcatacccgttattcgtagagtaaaagggtatactagatgtgtttccgaccatgtaaagtatatatattcttgatcaggatcaatagtcgagtcgatctggccctgtccgtatgaatgtctcgatctcaggaactataaaagctagaaggttgagattaagcatataaattctagagacatagatgcagcgcttggttgtttacccatgttgccacgcccacttaccgcccaaaacttccacgcccacaattttaaattttttctcattttatttcccaatatctcttggatatcccagaaaaatgatgaaatttcgcgttcgtatttccactagctgagtaacgggtatctgatagtcgggaaattcgactttagcattctctcttgtttttaacttgtggtttcgttatgctatatattcccccactcaaacaacttccactcaaatcaactcccaaatatcttttaggagcattctacaatctgatttttgtaatcatccagcaaacgtttccaaaactcaatttttttttaatacgtattaagccaaaagtcgtatacataactatttaaagcaattctgcagctgcagcaaagataatctatttaagagtaaagcattagtcaaaactaaagattattttcgttcaacgaacagcgaattatagattgctttgcccaaaatgtggatgctgtgagctaaaaaaaacctttttttttaataggctaagacatttttttgaataggctaagactttttttgagcatgaatttttttgagcacgtgaacctaggattaagaacaacaattcaagtaagccatatatacccatattatatatgcgaacatataactattaaaatattcaaataaaaatgagcattgctactacag

SEQ ID NO: 93 - RNA, 435 nt, synthetic construct
  source 1..435: mol_type = other RNA
ggaaaagtaaggaaaacgattccttctaacagaaatgtcctgagcaatcacctatgaacttgtttcaaatgcatgatcaaatgcaacctcacaaccttggctgagtcttgagactgaaagatttagccataatgtaaactgcctcaaattggactttgggcataaaagaacttttttatgcttaccatcttttttttttctttaacagatttgtatttaagaattgtttttaaaaaattttaagatttacacaatgtttctctgtaaatattgccattaaatgtaaataactttaataaaacgtttatagcagttacacagaatttcaatcctagtatatagtacctagtattataggtactataaaccctaattttttttatttaagtacattttgctttttaaagttgatttttttctattgtttttagaaaa

SEQ ID NO: 94 - RNA, 26 nt, synthetic construct
  source 1..26: mol_type = other RNA
aggtcagagtggaccccgtcatgggg

SEQ ID NO: 95 - RNA, 780 nt, synthetic construct
  source 1..780: mol_type = other RNA
gggggcagggaaggggaggcagccggcacccacaagtgccactgcccgagctggtgcattacagagaggagaaacacatcttccctagagggttcctgtagacctagggaggaccttatctgtgcgtgaaacacaccaggctgtgggcctcaaggacttgaaagcatccatgtgtggactcaagtccttacctcttccggagatgtagcaaaacgcatggagtgtgtattgttcccagtgacacttcagagagctggtagttagtagcatgttgagccaggcctgggtctgtgtctcttttctctttctccttagtcttctcatagcattaactaatctattgggttcattattggaattaacctggtgctggatattttcaaattgtatctagtgcagctgattttaacaataactactgtgttcctggcaatagtgtgttctgattagaaatgaccaatattatactaagaaaagatacgactttattttctggtagatagaaataaatagctatatccatgtactgtagtttttcttcaacatcaatgttcattgtaatgttactgatcatgcattgttgaggtggtctgaatgttctgacattaacagttttccatgaaaacgttttattgtgtttttaatttatttattaagatggattctcagatatttatatttttattttatttttttctaccttgaggtcttttgacatgtggaaagtgaatttgaatgaaaaatttaagcattgtttgcttattgttccaagacattgtc

SEQ ID NO: 96 - RNA, 336 nt, unidentified
  source 1..336: mol_type = other RNA
cggctgggggcacagtgggctgggcgcccctgcagaacatgaaccttccgctcctggctgccacagggtcctccgatgctggcctttgcgcctctagaggcagccactcatggattcaagtcctggctccgcctcttccatcaggaccactattaagccataggagtcctgggggtgcaaagggtgcccctctgtcaacacccttggctcctgtgtttagaggggtggcctgaaggaccttttctgctgggacaagacactgtactgccctctgctgggaaggggttttaataaacagaccctggcgcttgtgatgtaaaaaaaaaaaaaaaaaaa

SEQ ID NO: 97 - RNA, 1028 nt, synthetic construct
  source 1..1028: mol_type = other RNA
gttgggttcttaatcaagatacatatatgcaaattttgactgggctggcaccggaaccgacaaaataagaactttttgatgattttacgatttacgctgatggatcgctgcttttacggaattcgcttagttttaatatgttttatatgtagtatgttctctgtctttgtttatttatatgttcgtgcacttgtcctagtccattattgtatattattgtgtgttttgtgttctatgttagatttaaacttctcaatttttcgctgtctgtgatttgttttgccaatgccattgattttctgcacactttttgctgctatcccaaaagctgtgtaaaataatcaaatgcaaaataagcgcaagcagctgaaaacttctcttcaaacttttccgcttttcccaaaaccattttgctttgaaatctgtttttaccaaatcagattaaactgcaaaatggaacttaaatgcaaatcattgcaatgcttataaactgttttttgttctatatacttttgtgtgggtcaaaattcggcatgctcctgtatcacacaacctgccacttgcccttaaaaagaagggcgcagtgggcgtggtacgtatacatatgagccatgctgcattttggccgtaatgaaaatgcactgctttacttggaaaattcgcttgcacaaaatcaacgccgcggctgatttattattgatgtgctcaagcaaattcaagtgaagcatttgcgcgattttcgtctttctgtttccgtttgcaaaaaagtttataaaatgcttacactctgctgcagacacgccaaccggaagtgcgcactaagcgcttgtttgtagcacagtgtagaattctggcgtaatttacagctctactttaaagtcttctagatagctatctactatttataaacttatttattgtcttgaatgtatgttaattgtatgtattgatggtgatcacgttttttttgtcctataacaagctgcaatgtaaaatccaaaaaaaaaatgaaaaaataaaataaaagg

SEQ ID NO: 98 - RNA, 248 nt, synthetic construct
  source 1..248: mol_type = other RNA
aaaaacagatcaaatcttcagctattgctagtcgcacccaaccataacacacatcaaaccattgattggccaacaagtattacctcagccacaaagtatttatattccctagaactacctttttgccttataaattagtatttaaggttttatatagtttctaaggatagtttctaatggaagacaatttatatttaagtttttttttatagcatacattgaggacattaaactgatatatataaaat

SEQ ID NO: 99 - RNA, 357 nt, synthetic construct
  source 1..357: mol_type = other RNA
tcggatatagtaccatatatatagccacattatgggatcgtgcaagaatcggacggatttgtgtaatattaaatgtagccgtttagcgcgttaagtaacttcaagtttcattcaagttatgcatatatgtatctaagagtatatagagtaccagatcaaatgtttctcctctgacaactgcaatgtaagcttaggctaaaaaaaaacttaaaaatactaaacttaattagcgcaataagattgtaaactgtgatacgtttttcattgtctaacagacttcacactaaacacttcgtctatatgaaacacataatctaaataattttaaatcgtttaataaaattctttataatcatg

SEQ ID NO: 100 - RNA, 214 nt, synthetic construct
  source 1..214: mol_type = other RNA
tcgaggaaaatgggaaatccgaaaaaaaataccactttccaatcagctttaaagactccaacggattcggtctctaaacatcatccgcaacagctttaactctccacactgtgcaagtggagattttaaaatgaaatgcacaaatatccagctttaatcattgtcttccatctatgtttaagagagtatgaataaatacataatattaataccg

SEQ ID NO: 101 - RNA, 951 nt, synthetic construct
  source 1..951: mol_type = other RNA
gcttcctaggacccctgactcacgacctcatcaacgttggtgctactgcttggtggagaatgtaaaccctttgtaaccccatcccatgcccctccgactccccaccccaggagggaacgggcaggccgggcggccttgcagatccacagggcaaggaaacaagaggggagcggccaagtgccccgaccaggaggccccctacttcagaggcaagggccatgtggtcctggccccccaccccatcccttcccacctaggagctccccctccacacagcctccatctccaggggaacttggtgctacacgctggtgctcttatcttcctggggggagggaggagggaagggtggcccctcggggaaccccctacctggggctcctctaaagatggtgcagacacttcctgggcagtcccagctccccctgcccaccaggacccaccgttggctgccatccagttggtacccaagcacctgaagcctcaaagctggattcgctctagcatccctcctctcctgggtccacttggccgtctcctccccaccgatcgctgttccccacatctggggcgcttttgggttggaaaaccaccccacactgggaatagccaccttgcccttgtagaatccatccgcccatccgtccattcatccatcggtccgtccatccatgtccccagttgaccgcccggcaccactagctggctgggtgcacccaccatcaacctggttgacctgtcatggccgcctgtgccctgcctccacccccatcctacactcccccagggcgtgcggggctgtgcagactggggtgccaggcatctcctccccacccggggtgtccccacatgcagtactgtataccccccatccctccctcggtccactgaacttcagagcagttcccattcctgccccgcccatctttttgtgtctcgctgtgatagatc

SEQ ID NO: 102 - RNA, 56 nt, synthetic construct
  source 1..56: mol_type = other RNA
gtccaccactccccgcccacccctctgcaatgaataaagcctttgaatgagcacca

SEQ ID NO: 103 - RNA, 540 nt, synthetic construct
  source 1..540: mol_type = other RNA
accggactgttaccaacacccacacccctgtgatgaaacaaaacccataaatgcgcataaaacaagacgagattggcatggctttatttgttttttcttttggcgcttgactcaggattaaaaaactggaatggtgaaggtgtcagcagcagtcttaaaatgaaacatgttggagcgaacgcccccaaagttctacaatgcatctgaggactttgattgtacatttgtttcttttttaatagtcattccaaatattgttataatgcattgttacaggaagttactcgcctctgtgaaggcaacagcccagctgggaggagccggtaccaattactggtgttagatgataattgcttgtctgtaaattatgtaacccaacaagtgtctttttgtatcttccgccttaaaaacaaaacacacttgatcctttttggtttgtcaagcaagcgggctgtgttccccagtgatagatgtgaatgaaggctttacagtcccccacagtctaggagtaaagtgccagtatgtgggggagggaggggg

SEQ ID NO: 104 - RNA, 585 nt, synthetic construct
  source 1..585: mol_type = other RNA
actttaagaaacggctttccacgttgcccccacctgaaccctgtctctcctgccctttctcagatccactctgaagtttcctctcctgtcctgctcacgtgtgtgagcctgtcctctcctacctatgagccctctctctctgtgtggcaaacattaaaaaaaaaaaaaagcaggaaagatcccaagtccaacagtgtggcttaaacatttgtttcttggtgttgttatggcgagtttttggtaatgatgatgcagtcatcttgggaaattcttgcactgtaccccggttttttgatctggtgcgtgtggccctgtgggagtccactttcctctctatttctctctgttccaagtgtgtgtgtgcaatgttccgttctgaggagtccaaaatattaagtgaattcaaaaaaccatttctgtttcctcattttcaatgtgatggaatgaacaaaaaggttaaaaaaattaaaaaaaaaacggtttgttttaaaaataaataaataaagcaaatgtgccaattagcgtaacttaaggctgtgaggctcctttttcaatctgaatattaataaatcatgagagtaatca

SEQ ID NO: 105 - RNA, 85 nt, synthetic construct
  source 1..85: mol_type = other RNA
tagggtagtcaggtgctttgtgcttgtacatagtcttgtgttgctgtgtttgctgtaataaattattttgtagtgaaagtaccta

SEQ ID NO: 106 - RNA, 103 nt, synthetic construct
  source 1..103: mol_type = other RNA
atgaaataaattggtgataagtggaaaaaagagaaaaaccaatgattcataacaatgtatgtgaaagtgtaaaatagaatgttactttggaatgactataaac

SEQ ID NO: 107 - RNA, 152 nt, synthetic construct
  source 1..152: mol_type = other RNA
ggtctatgaacaaaatgcctcctgagcacttttatcactttgcttgaatatgcaaaatgcacttcttgtaaataactttttaagtcgtcgctggtttaaagttttactatgacctaatcaaatgattttgtaataaatgaacattgctatca

SEQ ID NO: 108 - RNA, 152 nt, synthetic construct
  source 1..152: mol_type = other RNA
atgcacagaatagcaagtccatcaaaactcctgcgtgagaattttaccagacttcaagagcatctcgccacatcttgaaaaatgccaccgtccgatgaaaaacaggagcctgctaaggaacaatgccacctgtcaataaatgttgaaaactc

SEQ ID NO: 109 - RNA, 197 nt, synthetic construct
  source 1..197: mol_type = other RNA
ggccctctgccacccaggcaggccctgccttcagccctggcccagagctggaacactctctgagatgcccctctgcctgggcttatgccctcagatggagacattggatgtggagctcctgctggatgcgtgccctgacccctgcaccagcccttccctgctttgaggacaaagagaataaagacttcatgttcaca

SEQ ID NO: 110 - RNA, 224 nt, synthetic construct
  source 1..224: mol_type = other RNA
aaacagatatgatcagatcactgttctagacagcatagggcaacaatattacatgctgctaatgtgttcaccttctattaagtgccagtagttctatgaccaacctttattgctagctgtgatacctacaattttaattgagtattttgattctactttattcatctaagagctcttttaataattctatttctattgattccaaataaatgaagttaagtatt

SEQ ID NO: 111 - RNA, 238 nt, synthetic construct
  source 1..238: mol_type = other RNA
atgctgacgtattctagaccgtgctgagcaataacatatgctgctatcctttcaagctccacgaagatcaccaagtgctaattcttctactgtaataaaagtttgaaatttgattccacttttgctcatttaaggtctcttccaatgattccatttcaatatattcttctttttaaagtattacacatttccacttctctccttaaatataaataaagtttaatgatcatgaaccaaa

SEQ ID NO: 112 - RNA, 301 nt, synthetic construct
  source 1..301: mol_type = other RNA
ttttttaaaagaaatcttcatttattcttcttttccaattgaactttcacatagcacagaaaaaattcaaactgcctatattgataaaaccatacagtgagccagccttgcagtaggcagtagactataagcagaagcacatatgaactggacctgcaccaaagctggcaccagggctcggaaggtctctgaactcagaaggatggcattttttgcaagttaaagaaaatcaggatctgagttattttgctaaacttgggggaggaggaacaaataaatggagtctttattgtgtatcata

SEQ ID NO: 113 - RNA, 261 nt, synthetic construct
  source 1..261: mol_type = other RNA
atggagccagtggatcctaggctggagccctggaagcacccaggctcccagcctaagaccgcctgcaccaactgctactgcaagaagtgctgcttccactgccaggtgtgcttcatcaccaaggccctgggcatcagctacggccggaagaagcggaggcagaggaggcggcccccccagggcagccagacccaccaggtgagcctgtccaagcagcccaccagccagtccaggggcgaccccaccggccccaaggagtga

SEQ ID NO: 114 - RNA, 321 nt, synthetic construct
  source 1..321: mol_type = other RNA
atggagacccccgcccagctgctgttcctgctgctgctgtggctgcccgacaccaccggcatggagccagtggatcctaggctggagccctggaagcacccaggctcccagcctaagaccgcctgcaccaactgctactgcaagaagtgctgcttccactgccaggtgtgcttcatcaccaaggccctgggcatcagctacggccggaagaagcggaggcagaggaggcggcccccccagggcagccagacccaccaggtgagcctgtccaagcagcccaccagccagtccaggggcgaccccaccggccccaaggagtga

SEQ ID NO: 115 - RNA, 306 nt, synthetic construct
  source 1..306: mol_type = other RNA
atgtggctggtgagcctggccatcgtgaccgcctgcgccggcgccatggagccagtggatcctaggctggagccctggaagcacccaggctcccagcctaagaccgcctgcaccaactgctactgcaagaagtgctgcttccactgccaggtgtgcttcatcaccaaggccctgggcatcagctacggccggaagaagcggaggcagaggaggcggcccccccagggcagccagacccaccaggtgagcctgtccaagcagcccaccagccagtccaggggcgaccccaccggccccaaggagtga

SEQ ID NO: 116 - RNA, 309 nt, synthetic construct
  source 1..309: mol_type = other RNA
atgttcgtgttcctggtgctgctgcccctggtgagcagccagtgcgtgatggagccagtggatcctaggctggagccctggaagcacccaggctcccagcctaagaccgcctgcaccaactgctactgcaagaagtgctgcttccactgccaggtgtgcttcatcaccaaggccctgggcatcagctacggccggaagaagcggaggcagaggaggcggcccccccagggcagccagacccaccaggtgagcctgtccaagcagcccaccagccagtccaggggcgaccccaccggccccaaggagtga

SEQ ID NO: 117 - RNA, 342 nt, synthetic construct
  source 1..342: mol_type = other RNA
atggagttcggcctgagctgggtgttcctggtggccatcctgaagggcgtgcagtgcgaggtgcagctgctggagagcggcatggagccagtggatcctaggctggagccctggaagcacccaggctcccagcctaagaccgcctgcaccaactgctactgcaagaagtgctgcttccactgccaggtgtgcttcatcaccaaggccctgggcatcagctacggccggaagaagcggaggcagaggaggcggcccccccagggcagccagacccaccaggtgagcctgtccaagcagcccaccagccagtccaggggcgaccccaccggccccaaggagtga

SEQ ID NO: 118 - RNA, 330 nt, synthetic construct
  source 1..330: mol_type = other RNA
atggacgccatgaagaggggcctgtgctgcgtgctgctgctgtgcggcgccgtgttcgtgagccccagcatggagccagtggatcctaggctggagccctggaagcacccaggctcccagcctaagaccgcctgcaccaactgctactgcaagaagtgctgcttccactgccaggtgtgcttcatcaccaaggccctgggcatcagctacggccggaagaagcggaggcagaggaggcggcccccccagggcagccagacccaccaggtgagcctgtccaagcagcccaccagccagtccaggggcgaccccaccggccccaaggagtga

SEQ ID NO: 119 - RNA, 315 nt, synthetic construct
  source 1..315: mol_type = other RNA
atgaagtgggtgaccttcatcagcctgctgttcctgttctccagcgcctacagcatggagccagtggatcctaggctggagccctggaagcacccaggctcccagcctaagaccgcctgcaccaactgctactgcaagaagtgctgcttccactgccaggtgtgcttcatcaccaaggccctgggcatcagctacggccggaagaagcggaggcagaggaggcggcccccccagggcagccagacccaccaggtgagcctgtccaagcagcccaccagccagtccaggggcgaccccaccggccccaaggagtga

SEQ ID NO: 120 - RNA, 306 nt, synthetic construct
  source 1..306: mol_type = other RNA
atggagcccgtggacccccggctggagccctggaagcaccccggcagccagcccaagaccgccagcaacaactgctactgcaagcggtgctgcctgcactgccaggtgtgcttcaccaagaagggcctgggcatcagctacggcaggaagaagcggcggcagaggaggcgggccccccaggactccaagacccaccaggtgagcctgagcaagcagcccgcctcccagcccaggggcgaccccaccggccccaaggagagcaagaagaaggtggagcgggagaccgagaccgaccccgaggactga

SEQ ID NO: 121 - RNA, 360 nt, synthetic construct
  source 1..360: mol_type = other RNA
atggactggacctggatcctgttcctggtggccgccgccaccagggtgcactccatggagcccgtggacccccggctggagccctggaagcaccccggcagccagcccaagaccgccagcaacaactgctactgcaagcggtgctgcctgcactgccaggtgtgcttcaccaagaagggcctgggcatcagctacggcaggaagaagcggcggcagaggaggcgggccccccaggactccaagacccaccaggtgagcctgagcaagcagcccgcctcccagcccaggggcgaccccaccggccccaaggagagcaagaagaaggtggagcgggagaccgagaccgaccccgaggactga

SEQ ID NO: 122 - RNA, 366 nt, synthetic construct
  source 1..366: mol_type = other RNA
atggagacccccgcccagctgctgttcctgctgctgctgtggctgcccgacaccaccggcatggagcccgtggacccccggctggagccctggaagcaccccggcagccagcccaagaccgccagcaacaactgctactgcaagcggtgctgcctgcactgccaggtgtgcttcaccaagaagggcctgggcatcagctacggcaggaagaagcggcggcagaggaggcgggccccccaggactccaagacccaccaggtgagcctgagcaagcagcccgcctcccagcccaggggcgaccccaccggccccaaggagagcaagaagaaggtggagcgggagaccgagaccgaccccgaggactga

SEQ ID NO: 123 - RNA, 351 nt, synthetic construct
  source 1..351: mol_type = other RNA
atgtggctggtgagcctggccatcgtgaccgcctgcgccggcgccatggagcccgtggacccccggctggagccctggaagcaccccggcagccagcccaagaccgccagcaacaactgctactgcaagcggtgctgcctgcactgccaggtgtgcttcaccaagaagggcctgggcatcagctacggcaggaagaagcggcggcagaggaggcgggccccccaggactccaagacccaccaggtgagcctgagcaagcagcccgcctcccagcccaggggcgaccccaccggccccaaggagagcaagaagaaggtggagcgggagaccgagaccgaccccgaggactga

SEQ ID NO: 124 - RNA, 354 nt, synthetic construct
  source 1..354: mol_type = other RNA
atgttcgtgttcctggtgctgctgcccctggtgagcagccagtgcgtgatggagcccgtggacccccggctggagccctggaagcaccccggcagccagcccaagaccgccagcaacaactgctactgcaagcggtgctgcctgcactgccaggtgtgcttcaccaagaagggcctgggcatcagctacggcaggaagaagcggcggcagaggaggcgggccccccaggactccaagacccaccaggtgagcctgagcaagcagcccgcctcccagcccaggggcgaccccaccggccccaaggagagcaagaagaaggtggagcgggagaccgagaccgaccccgaggactga

SEQ ID NO: 125 - RNA, 387 nt, synthetic construct
  source 1..387: mol_type = other RNA
atggagttcggcctgagctgggtgttcctggtggccatcctgaagggcgtgcagtgcgaggtgcagctgctggagagcggcatggagcccgtggacccccggctggagccctggaagcaccccggcagccagcccaagaccgccagcaacaactgctactgcaagcggtgctgcctgcactgccaggtgtgcttcaccaagaagggcctgggcatcagctacggcaggaagaagcggcggcagaggaggcgggccccccaggactccaagacccaccaggtgagcctgagcaagcagcccgcctcccagcccaggggcgaccccaccggccccaaggagagcaagaagaaggtggagcgggagaccgagaccgaccccgaggactga

SEQ ID NO: 126 - RNA, 360 nt, synthetic construct
  source 1..360: mol_type = other RNA
atggactggacctggatcctgttcctggtggccgccgccaccagggtgcacagcatggagcccgtggaccccaggctggagccctggaagcaccccggcagccagcccaagaccgccagcaacaactgctactgcaagaggtgctgcctgcactgccaggtgtgcttcaccaagaagggcctgggcatcagctacggcaggaagaagaggaggcagaggaggagagccccccaggacagcaagacccaccaggtgagcctgagcaagcagcccgccagccagcccaggggcgaccccaccggccccaaggagagcaagaagaaggtggagcgggagaccgagaccgaccccgaggactga

SEQ ID NO: 127 - RNA, 393 nt, synthetic construct
  source 1..393: mol_type = other RNA
atggagacacccttgagggagcaggagaactcattagaatcctccaacgagcgctcttcatgcatttcagaggcggatgcatccactccagaatcggccaacctgggggaggaaatcctctctcagctataccgccctctagaagcatgctataacacatgctattgtaaaaagtgttgctaccattgccagttttgttttcttaaaaaaggcttggggatatgttatgagcaatcacgaaagagaagaagaactccgaaaaaggctaaggctaatacatcttctgcatcaaacaaacccatatccaacaggacccggcactgccaaccagagaaggcaaagaaagagacggtggagaaggcggtggcaacagctcctggccttggcagatag

SEQ ID NO: 128 - RNA, 447 nt, synthetic construct
  source 1..447: mol_type = other RNA
atggactggacctggatcctcttcttggtggcagcagccacgcgagtccactccatggagacacccttgagggagcaggagaactcattagaatcctccaacgagcgctcttcatgcatttcagaggcggatgcatccactccagaatcggccaacctgggggaggaaatcctctctcagctataccgccctctagaagcatgctataacacatgctattgtaaaaagtgttgctaccattgccagttttgttttcttaaaaaaggcttggggatatgttatgagcaatcacgaaagagaagaagaactccgaaaaaggctaaggctaatacatcttctgcatcaaacaaacccatatccaacaggacccggcactgccaaccagagaaggcaaagaaagagacggtggagaaggcggtggcaacagctcctggccttggcagatag

SEQ ID NO: 129 - protein, 101 aa, Human immunodeficiency virus 1
MDPVDPSLEPWNHPGSQPKTPCNKCYCKVCCYHCQCCFLNKGLGISYGRKKRKPRRGTPQSNKDHQNPIPKQPIPRTQGDSTGPEESKKKVESKTEADRYA

SEQ ID NO: 130 - protein, 101 aa, Human immunodeficiency virus 1
MEPVDPKLEPWNHPGSQPKTACTKCYCKRCCYHCQLCFINKGLGISYGRKKRRPRRKPSPSNKDHQNPIPKQSLPQAQRVPTGPEEPKKEVESKAETDRFD

SEQ ID NO: 131 - protein, 100 aa, Human immunodeficiency virus 1
MEPVDPRLEPWKHPGSQPKTACTNCYCKKCCFHCQVCFITKALGISYGRKKRRQRRRAHQNSQTHQASLSKQPTSQPRGDPTGPKEKKKVERETETDPFD

SEQ ID NO: 132 - protein, 86 aa, Human immunodeficiency virus 1
MEPVDPRLEPWKHPGSQPKTACTNCYCKKCCFHCQVCFITKALGISYGRKKRRQRRRAHQNSQTHQASLSKQPTSQPRGDPTGPKE

SEQ ID NO: 133 - protein, 101 aa, Human immunodeficiency virus 1
MEPVDPRLEPWKHPGSQPKTASNNCYCKRCCLHCQVCFTKKGLGISYGRKKRRQRRRAPQDSKTHQVSLSKQPASQPRGDPTGPKESKKKVERETETDPED

SEQ ID NO: 134 - protein, 86 aa, Human immunodeficiency virus 1
MEPVDPRLEPWKHPGSQPKTACTNCYCKKCCFHCQVCFITKALGISYGRKKRRQRRRPPQGSQTHQVSLSKQPTSQSRGDPTGPKE

SEQ ID NO: 135 - protein, 101 aa, Human immunodeficiency virus 1
MEPVDPRLEPWKHPGSQPKTACNNCYCKRCCLHCQVCFTKKGLGISYGRKKRRQRRRAPQDSKTHQVSLSKQPASQPRGDPTGPKESKKKVERETETDPED

SEQ ID NO: 136 - protein, 101 aa, Human immunodeficiency virus 1
MEPVDPSLEPWKHPGSQPKTACNTCYCKRCCFHCQVCFITKGLGISYGRKKRRQRRRAPRDSQSHQASLSKQPTSQPRGDPTSPKEPKKKVEKEAETDPGV

SEQ ID NO: 137 - protein, 101 aa, Human immunodeficiency virus 1
MEPVDPRLEPWKHPGSQPKTACTNCYCKKCCFHCQVCFTKKGLGISYGRKKRRQRRRSHPDSKIHQAPLSTQPTSQPRGDPTGPKESKEKVERETETDRVD

SEQ ID NO: 138 - protein, 101 aa, Human immunodeficiency virus 1
MEPVDPSLEPWKHPGSQPKTACTNCYCKRCCFHCQVCFTKKALGISYGRKKRRQRRRAPQDSETXQASLSKQPTSQXGGDXTGPKESKKKVETTTETDPLY

SEQ ID NO: 139 - protein, 101 aa, Human immunodeficiency virus 1
MEPVDPRLEPWKHPGSQPRTPCNNCYCKQCCFHCQVCFTKKGLGISYGRKKRRQRRRAHQDSETHQADLSKQPTSQQRGDPTGPKESKKKVEREAETDPCD

SEQ ID NO: 140 - protein, 86 aa, Human immunodeficiency virus 1
MEPVDPRLEPWKHPGSQPKTACTNCYCKKCCFHCQVCFSRKGLGISYGRKKRRQRRRAPKDSETHQANLSKQPSSQLRGDPTGPKE

SEQ ID NO: 141 - protein, 101 aa, Human immunodeficiency virus 1
MEPVDPRLEPWKHPGSQPRTACTKCYCKKCCFHCQVCFMTKGLGISYGRKKRRQRRRPPQDSEAHQVPLPKQPASQPRGDPTGPKESKEKVESKTETDPDH

SEQ ID NO: 142 - protein, 101 aa, Human immunodeficiency virus 1
MEPVDPRLEPWKHPGSQPRTACTNCYCKKCCFHCQMCFMKKGLGISYGRKKRRQRRGSPQDSQTHQISLPKQPASQHRGDPTGPEKPKKKVERETETDPTD

SEQ ID NO: 143 - protein, 101 aa, Human immunodeficiency virus 1
MDPVDPRLEPWKHPGSQPRTXCXNCYCKKCCXHCQVCFXKKALGISYGRKKRRQRRRADQDSQXHQVSLSKQPASQPSGDPTGQKESKKKVETETKADPVD

SEQ ID NO: 144 - protein, 102 aa, Human immunodeficiency virus 1
MELVDPRLEPWKHPGSQPRTACXNCYCKXCCYHCQVCFLTKGLGISYGRKKRRQRRRXSQBSQTHQAALSKQPASQPRGDPKGPKEQKKKVERETETDPQDW

SEQ ID NO: 145 - protein, 101 aa, Human immunodeficiency virus 1
MDPVDPRLEPWKHPGSQPRTPCTKCYCKSCCFHCQVCFITKGLGISYGRKKRRPRRRAPEGSSTHQISISEQPTPQPRGDPTGPKESKKKVERETETDQFD

SEQ ID NO: 146 - protein, 101 aa, Human immunodeficiency virus 1
MEPVDPRLEPWKHPGSQPKTACNNCYCKKCCFHCQVCFTRKGLGISYGRKKRRQRRRTPQDSQTHQVSLSKQPTSQLRGDPTGPKESKKKVERETETDPGH

SEQ ID NO: 147 - protein, 101 aa, Human immunodeficiency virus 1
MEPIDPSLEPWKHPGSQPETPCTNCYCKKCCFHCQVCFIKKALGISYGRKKRRQRRRAPQTSQTHQGSLSKQPTSQSRGDPTGPKESKKKVERETETDPED

SEQ ID NO: 148 - protein, 101 aa, Human immunodeficiency virus 1
MEPVDPRLEPWKHPGSQPRTACNNCYCKQCCFHCQVCFITKGLGICYGRKKRRQRRRAPRDSQIHQVSLPKQPSSQLRGDPTGPTEPKEKVERETETDLCD

SEQ ID NO: 149 - protein, 101 aa, Human immunodeficiency virus 1
MEPVDPNLEPWNHPGSQPKTPCNNCYCKKCSYHCLVCFQTKGLGISYGRKKRRQRRRAPPSSEDHQNLISKQPLPQTRGDQTGSEESKKKVESKTETDPFD

SEQ ID NO: 150 - protein, 101 aa, Human immunodeficiency virus 1
MEPVDPNLEPWNHPGSQPKTACNTCYCKYCSYHCLVCFQTKGLGISYGRKKRRQRRSAPQSSEDHQNLISKQPLPRTQGDTTGSEESKKKVESKTKTDPFD

SEQ ID NO: 151 - protein, 101 aa, Human immunodeficiency virus 1
MEQVDPNLEPWNHPGSQPKTPCNKCFCKSCSYHCLVCFQTKGLGISYGRKKRRQRRHAPPGSKDHQNPISKQPLPQTRGDPTGSEESKKKVESKTETDPFD

SEQ ID NO: 152 - protein, 101 aa, Human immunodeficiency virus 1
MEPVDPNLEPWNHPGSQPKTACNKCFCKKCSYHCLVCFQKKGLGISYGRKKRRQRRSAPPSSEDHQNPVSKQPLSQTRGDPTGSEESKKKVESKTETDQCD

SEQ ID NO: 153 - protein, 101 aa, Human immunodeficiency virus 1
MEPVDPNLEPWNHPGSQPKTACNNCFCKKCSYHCLVCFQTKGLGISYGRKKRRQRRSAPPSSEDHQIPISKQPLPQARGDQTGSEKSKKKVESKTETDPFD

SEQ ID NO: 154 - protein, 99 aa, Human immunodeficiency virus 1
MDPVDPNLEPWNHPGSQPRTPCNKCHCKKCCYHCPVCFLNKGLGISYGRKKRRQRRGPPQGGQAHQVPIPKQPSSQPRGDPTGPKEQKKKVESEAETDP

SEQ ID NO: 155 - protein, 86 aa, Human immunodeficiency virus 1
MEPVDHNLEPWNHPGSQPSTPRNKCYCKKCCYHCQVCFITKGLGISYGRKKWRQRRRSSQGGQAHQDPIPKQPSSQSRGNPTGPKE

SEQ ID NO: 156 - protein, 86 aa, Human immunodeficiency virus 1
MDPVDPNLEPWNHPGSQPRTPCNNCYCKKCCYHCQNCFITKGLGISYGRKKRRQRRRTPQGDQAHQDPIPKQPSSQPRGDQTGPKE

SEQ ID NO: 157 - protein, 101 aa, Human immunodeficiency virus 1
MELVDPNLEPWNHPGSQPTTACSKCYCKKCCWHCQLCFLKKGLGISYGRKKRKHRRGTPQSSKDHQNPIPKQPLPIIRRNPTDPKESKKEVASKAETDQCD

SEQ ID NO: 158 - protein, 99 aa, Human immunodeficiency virus 1
MKPVDPNLEPWNHPGSQPTTNCNTCYCKKCCWHCQLCFLKKGLGISYGRKKRKHRRGTPQSSKDHQNPIREQPLPIIRGNPTDPKESKKEGASKAETDP

SEQ ID NO: 159 - protein, 130 aa, Human immunodeficiency virus 2
METPLKAPESSLKSCNEPFSRTSEQDVATQELARQGEEILSQLYRPLETCNNSCYCKRCCYHCQMCFLNKGLGICYERKGRRRRTPKKTKTHPSPTPDKSISTRTGDSQPTKKQKKTVEATVETDTGPGR

SEQ ID NO: 160 - protein, 130 aa, Simian immunodeficiency virus
METPLREQENSLESSNERSSCISEADASTPESANLGEEILSQLYRPLEACYNTCYCKKCCYHCQFCFLKKGLGICYEQSRKRRRTPKKAKANTSSASNKPISNRTRHCQPEKAKKETVEKAVATAPGLGR

SEQ ID NO: 161 - protein, 18 aa, synthetic construct
MDWTWILFLVAAATRVHS

SEQ ID NO: 162 - protein, 20 aa, synthetic construct
METPAQLLFLLLLWLPDTTG

SEQ ID NO: 163 - protein, 15 aa, synthetic construct
MWLVSLAIVTACAGA

SEQ ID NO: 164 - protein, 16 aa, synthetic construct
MFVFLVLLPLVSSQCV

SEQ ID NO: 165 - protein, 23 aa, synthetic construct
MDAMKRGLCCVLLLCGAVFVSPS

SEQ ID NO: 166 - protein, 18 aa, synthetic construct
MKWVTFISLLFLFSSAYS

SEQ ID NO: 167 - protein, 27 aa, synthetic construct
MEFGLSWVFLVAILKGVQCEVQLLESG

SEQ ID NO: 168 - protein, 106 aa, synthetic construct
METPAQLLFLLLLWLPDTTGMEPVDPRLEPWKHPGSQPKTACTNCYCKKCCFHCQVCFITKALGISYGRKKRRQRRRPPQGSQTHQVSLSKQPTSQSRGDPTGPKE

SEQ ID NO: 169 - protein, 101 aa, synthetic construct
MWLVSLAIVTACAGAMEPVDPRLEPWKHPGSQPKTACTNCYCKKCCFHCQVCFITKALGISYGRKKRRQRRRPPQGSQTHQVSLSKQPTSQSRGDPTGPKE

SEQ ID NO: 170 - protein, 102 aa, synthetic construct
MFVFLVLLPLVSSQCVMEPVDPRLEPWKHPGSQPKTACTNCYCKKCCFHCQVCFITKALGISYGRKKRRQRRRPPQGSQTHQVSLSKQPTSQSRGDPTGPKE

SEQ ID NO: 171 - protein, 113 aa, synthetic construct
MEFGLSWVFLVAILKGVQCEVQLLESGMEPVDPRLEPWKHPGSQPKTACTNCYCKKCCFHCQVCFITKALGISYGRKKRRQRRRPPQGSQTHQVSLSKQPTSQSRGDPTGPKE

SEQ ID NO: 172 - protein, 109 aa, synthetic construct
MDAMKRGLCCVLLLCGAVFVSPSMEPVDPRLEPWKHPGSQPKTACTNCYCKKCCFHCQVCFITKALGISYGRKKRRQRRRPPQGSQTHQVSLSKQPTSQSRGDPTGPKE

SEQ ID NO: 173 - protein, 104 aa, synthetic construct
MKWVTFISLLFLFSSAYSMEPVDPRLEPWKHPGSQPKTACTNCYCKKCCFHCQVCFITKALGISYGRKKRRQRRRPPQGSQTHQVSLSKQPTSQSRGDPTGPKE

SEQ ID NO: 174 - protein, 119 aa, synthetic construct
MDWTWILFLVAAATRVHSMEPVDPRLEPWKHPGSQPKTASNNCYCKRCCLHCQVCFTKKGLGISYGRKKRRQRRRAPQDSKTHQVSLSKQPASQPRGDPTGPKESKKKVERETETDPED

SEQ ID NO: 175 - protein, 121 aa, synthetic construct
METPAQLLFLLLLWLPDTTGMEPVDPRLEPWKHPGSQPKTASNNCYCKRCCLHCQVCFTKKGLGISYGRKKRRQRRRAPQDSKTHQVSLSKQPASQPRGDPTGPKESKKKVERETETDPED

SEQ ID NO: 176 - protein, 116 aa, synthetic construct
MWLVSLAIVTACAGAMEPVDPRLEPWKHPGSQPKTASNNCYCKRCCLHCQVCFTKKGLGISYGRKKRRQRRRAPQDSKTHQVSLSKQPASQPRGDPTGPKESKKKVERETETDPED

SEQ ID NO: 177 - protein, 117 aa, synthetic construct
MFVFLVLLPLVSSQCVMEPVDPRLEPWKHPGSQPKTASNNCYCKRCCLHCQVCFTKKGLGISYGRKKRRQRRRAPQDSKTHQVSLSKQPASQPRGDPTGPKESKKKVERETETDPED

SEQ ID NO: 178 - protein, 128 aa, synthetic construct
MEFGLSWVFLVAILKGVQCEVQLLESGMEPVDPRLEPWKHPGSQPKTASNNCYCKRCCLHCQVCFTKKGLGISYGRKKRRQRRRAPQDSKTHQVSLSKQPASQPRGDPTGPKESKKKVERETETDPED

SEQ ID NO: 179 - protein, 148 aa, synthetic construct
MDWTWILFLVAAATRVHSMETPLREQENSLESSNERSSCISEADASTPESANLGEEILSQLYRPLEACYNTCYCKKCCYHCQFCFLKKGLGICYEQSRKRRRTPKKAKANTSSASNKPISNRTRHCQPEKAKKETVEKAVATAPGLGR

SEQ ID NO: 180 - DNA, 31 bp, synthetic construct
  source 1..31: mol_type = other DNA
tgccaagctttaatacgactcactataggga

SEQ ID NO: 181 - DNA, 103 bp, synthetic construct
  source 1..103: mol_type = other DNA
ttttttttttttttttttttttttttttttttttttttttttttttttttttttttttttttttttttttttttttttttgctagctcagactttattcaaag

SEQ ID NO: 182 - protein, 101 aa, Human immunodeficiency virus 1
MEPVDPRLEPWKHPGSQPKTASNNCYCKRCCLHCQVCFTKKGLGISYGRKKHHQRRRAPQDSKTHQVSLSKQPASQPRGDPTGPKESKKKVERETETDPED

SEQ ID NO: 183 - protein, 20 aa, synthetic construct
MARPLCTLLLLMATLAGALA

SEQ ID NO: 184 - protein, 23 aa, synthetic construct
MDAMKRGLCCVLLLCGAVFVSAR

SEQ ID NO: 185 - protein, 29 aa, synthetic construct
MNSFSTSAFGPVAFSLGLLLVLPAAFPAP

SEQ ID NO: 186 - protein, 35 aa, synthetic construct
MACLGFQRHKAQLNLATRTWPCTLLFFLLFIPVFC

SEQ ID NO: 187 - protein, 25 aa, synthetic construct
MGGAAARLGAVILFVVIVGLHGVRG

SEQ ID NO: 188 - protein, 55 aa, synthetic construct
IVGIVAGLAVLAVVVIGAVVATVMCRRKSSGGKGGSYSQAASSDSAQGSDVSLTA

SEQ ID NO: 189 - protein, 27 aa, synthetic construct
GYIPEAPRDGQAYVRKDGEWVLLSTFL

SEQ ID NO: 190 - protein, 119 aa, synthetic construct
MDWTWILFLVAAATRVHSMEPVDPRLEPWKHPGSQPKTASNNCYCKRCCLHCQVCFTKKGLGISYGRKKHHQRRRAPQDSKTHQVSLSKQPASQPRGDPTGPKESKKKVERETETDPED

SEQ ID NO: 191 - protein, 174 aa, synthetic construct
MDWTWILFLVAAATRVHSMEPVDPRLEPWKHPGSQPKTASNNCYCKRCCLHCQVCFTKKGLGISYGRKKRRQRRRAPQDSKTHQVSLSKQPASQPRGDPTGPKESKKKVERETETDPEDIVGIVAGLAVLAVVVIGAVVATVMCRRKSSGGKGGSYSQAASSDSAQGSDVSLTA

SEQ ID NO: 192 - protein, 146 aa, synthetic construct
MDWTWILFLVAAATRVHSMEPVDPRLEPWKHPGSQPKTASNNCYCKRCCLHCQVCFTKKGLGISYGRKKRRQRRRAPQDSKTHQVSLSKQPASQPRGDPTGPKESKKKVERETETDPEDGYIPEAPRDGQAYVRKDGEWVLLSTFL

SEQ ID NO: 193 - protein, 121 aa, synthetic construct
MARPLCTLLLLMATLAGALAMEPVDPRLEPWKHPGSQPKTASNNCYCKRCCLHCQVCFTKKGLGISYGRKKRRQRRRAPQDSKTHQVSLSKQPASQPRGDPTGPKESKKKVERETETDPED

SEQ ID NO: 194 - protein, 124 aa, synthetic construct
MDAMKRGLCCVLLLCGAVFVSARMEPVDPRLEPWKHPGSQPKTASNNCYCKRCCLHCQVCFTKKGLGISYGRKKRRQRRRAPQDSKTHQVSLSKQPASQPRGDPTGPKESKKKVERETETDPED

SEQ ID NO: 195 - protein, 130 aa, synthetic construct
MNSFSTSAFGPVAFSLGLLLVLPAAFPAPMEPVDPRLEPWKHPGSQPKTASNNCYCKRCCLHCQVCFTKKGLGISYGRKKRRQRRRAPQDSKTHQVSLSKQPASQPRGDPTGPKESKKKVERETETDPED

SEQ ID NO: 196 - protein, 136 aa, synthetic construct
MACLGFQRHKAQLNLATRTWPCTLLFFLLFIPVFCMEPVDPRLEPWKHPGSQPKTASNNCYCKRCCLHCQVCFTKKGLGISYGRKKRRQRRRAPQDSKTHQVSLSKQPASQPRGDPTGPKESKKKVERETETDPED

SEQ ID NO: 197 - protein, 126 aa, synthetic construct
MGGAAARLGAVILFVVIVGLHGVRGMEPVDPRLEPWKHPGSQPKTASNNCYCKRCCLHCQVCFTKKGLGISYGRKKRRQRRRAPQDSKTHQVSLSKQPASQPRGDPTGPKESKKKVERETETDPED

SEQ ID NO: 198 - RNA, 360 nt, synthetic construct
  source 1..360: mol_type = other RNA
atggactggacctggatcctgttcctggtggccgccgccaccagggtgcacagcatggagcccgtggaccctcgcctggagccctggaagcaccctggcagccagcccaagaccgccagcaacaactgttactgcaagcggtgctgcctgcactgccaggtgtgcttcaccaagaagggcctgggcatctcctacggccggaagaagcaccaccagaggaggcgggcccctcaggactccaagacccaccaggtgagcctgagcaagcagcccgcctcccagccccggggcgaccccaccggccctaaggagagcaagaagaaggtggagcgggagaccgagaccgaccccgaggactga

SEQ ID NO: 199 - RNA, 360 nt, synthetic construct
  source 1..360: mol_type = other RNA
atggactggacctggatcctgttcctggtggccgccgccaccagggtgcacagcatggagcccgtggaccctaggctggagccctggaagcaccctggcagccagcccaagaccgccagcaacaactgttactgcaagcggtgctgcctgcactgccaggtgtgcttcaccaagaagggcctgggcatctcctacggcaggaagaagcaccaccagaggcggcgggccccccaggactccaagacccaccaggtgagcctgagcaagcagcctgccagccagcctcggggcgaccccaccggccccaaggagtccaagaagaaggtggagcgggagaccgagaccgaccccgaggactga

SEQ ID NO: 200 - RNA, 360 nt, synthetic construct
  source 1..360: mol_type = other RNA
atggactggacctggatcctgttcctggtggccgccgccaccagggtgcacagcatggagcctgtggacccccggctggagccctggaagcaccctggcagccagcccaagaccgccagcaacaactgttactgcaagcggtgctgcctgcactgccaggtgtgcttcaccaagaagggcctgggcatctcctacggcaggaagaagcaccaccagcggcggagggccccacaggactccaagacccaccaggtgagcctgagcaagcagcctgccagccagcctcggggcgaccccaccggccccaaggagtccaagaagaaggtggagcgggagaccgagaccgaccccgaggactga

SEQ ID NO: 201 - RNA, 360 nt, synthetic construct
  source 1..360: mol_type = other RNA
atggactggacctggatcctgttcctggtggccgccgccaccagggtgcacagcatggagcccgtggaccccaggctggagccctggaagcaccccggcagccagcccaagaccgccagcaacaactgctactgcaagaggtgctgcctgcactgccaggtgtgcttcaccaagaagggcctgggcatcagctacggcaggaagaagcaccaccagaggaggagggccccccaggacagcaagacccaccaggtgagcctgagcaagcagcccgccagccagcccaggggcgaccccaccggccccaaggagagcaagaagaaggtggagagggagaccgagaccgaccccgaggactga

SEQ ID NO: 202 - RNA, 360 nt, synthetic construct
  source 1..360: mol_type = other RNA
atggactggacctggatcctgttcctggtggccgccgccaccagggtgcacagcatggagcccgtggaccctcgcctggagccctggaagcaccctggcagccagcccaagaccgccagcaacaactgttactgcaagcggtgctgcctgcactgccaggtgtgcttcaccaagaagggcctgggcatctcctacggccggaagaagcggaggcagaggaggcgggcccctcaggacagcaagacccaccaggtgtccctgagcaagcagcccgcctcccagccccggggcgaccccaccggccctaaggagagcaagaagaaggtggagcgggagaccgagaccgaccccgaggactga

SEQ ID NO: 203 - RNA, 360 nt, synthetic construct; identical to SEQ ID NO: 126
  source 1..360: mol_type = other RNA

SEQ ID NO: 204 - RNA, 525 nt, synthetic construct
  source 1..525: mol_type = other RNA
atggactggacctggatcctgttcctggtggccgccgccaccagggtgcactccatggagcccgtggacccccggctggagccctggaagcaccccggcagccagcccaagaccgccagcaacaactgctactgcaagcggtgctgcctgcactgccaggtgtgcttcaccaagaagggcctgggcatctcttacggcaggaagaagcggcggcagaggaggcgggccccccaggacagcaagacccaccaggtgtccctgagcaagcagcccgcctcccagccccggggcgaccccaccggccccaaggagagcaagaagaaggtggagcgggagaccgagaccgaccccgaggacatcgtgggcatcgtggccggcctggccgtgctggccgtggtggtgatcggcgccgtggtggccaccgtgatgtgccggcggaagtccagcggcggcaagggcggcagctacagccaggccgccagcagcgacagcgcccagggctccgacgtgtccctgaccgcctga

SEQ ID NO: 205 - RNA, 441 nt, synthetic construct
  source 1..441: mol_type = other RNA
atggactggacctggatcctgttcctggtggccgccgccaccagggtgcactccatggagcccgtggacccccggctggagccctggaagcaccccggcagtcagcccaagaccgccagcaacaactgctactgcaagcggtgctgcctgcactgccaggtgtgcttcaccaagaagggcctgggcatcagctacggcaggaagaagcggaggcagaggaggcgggccccccaggacagcaagacccaccaggtgtccctgagcaagcagcccgcctcccagcccaggggcgaccccaccggccccaaggagagcaagaagaaggtggagcgggagaccgagaccgaccccgaggacggctacatccccgaggccccccgggacggccaggcctacgtgaggaaggacggcgagtgggtgctgctgagcaccttcctgtga

SEQ ID NO: 206 - RNA, 366 nt, synthetic construct
  source 1..366: mol_type = other RNA
atggcccggcccctgtgcaccctgctgctgctgatggccaccctggccggcgccctggccatggagcccgtggaccccaggctggagccctggaagcaccccggcagccagcccaagaccgccagcaacaactgctactgcaagcggtgctgcctgcactgccaggtgtgcttcaccaagaagggcctgggcatcagctacggcaggaagaagaggaggcagaggaggcgggcccctcaggacagcaagacccaccaggtgtccctgtccaagcagcccgccagccagcccaggggcgaccccaccggccccaaggagagcaagaagaaggtggagcgggagaccgagaccgaccccgaggactga

SEQ ID NO: 207 - RNA, 375 nt, synthetic construct
  source 1..375: mol_type = other RNA
atggacgccatgaagcggggcctgtgctgcgtgctgctgctgtgcggcgccgtgttcgtgtccgccaggatggagcccgtggaccccaggctggagccctggaagcaccccggcagccagcccaagaccgccagcaacaactgctactgcaagcggtgctgcctgcactgccaggtgtgcttcaccaagaagggcctgggcatcagctacggccggaagaagaggaggcagcggagacgcgccccccaggacagcaagacccaccaggtgagcctgagcaagcagcctgccagccagccccgtggcgaccccaccggccccaaggagagcaagaagaaggtggagcgggagaccgagaccgaccccgaggactga

SEQ ID NO: 208 - RNA, 393 nt, synthetic construct
  source 1..393: mol_type = other RNA
atgaactccttctccacctccgccttcggccccgtggccttcagcctgggcctgctgctggtgctgcccgccgccttccccgcccccatggagcccgtggaccccaggctggagccctggaagcaccccggcagccagcccaagaccgccagcaacaactgctactgcaagcggtgctgcctgcactgccaggtgtgcttcaccaagaagggcctgggcatcagctacggcaggaagaagaggaggcagaggaggagagccccccaggacagcaagacccaccaggtgagcctgtccaagcagcccgccagccagccccggggcgaccccaccggccccaaggagagcaagaagaaggtggagagggagaccgagaccgaccccgaggactga

SEQ ID NO: 209 - RNA, 411 nt, synthetic construct
  source 1..411: mol_type = other RNA
atggcctgcctgggctttcagcggcacaaggcccagctgaacctggccaccaggacctggccctgcaccctgctgttcttcctgctgttcatccccgtgttctgcatggagcccgtggacccccggctggagccctggaagcaccccggcagccagcccaagaccgccagcaacaactgctactgcaagaggtgctgcctgcactgccaggtgtgcttcaccaagaagggcctgggcatctcctacggcaggaagaagcggaggcagaggaggcgggccccccaggacagcaagacccaccaggtgtccctgagcaagcagcccgcctcccagccccggggcgaccccaccggccccaaggagagcaagaagaaggtggagcgggagaccgagaccgaccccgaggactga

SEQ ID NO: 210 - RNA, 381 nt, synthetic construct
  source 1..381: mol_type = other RNA
atgggcggcgccgccgccaggctgggcgccgtgatcctgttcgtggtgatcgtgggcctgcacggcgtgaggggcatggagcccgtggaccccaggctggagccctggaagcaccccggcagccagcccaagaccgccagcaacaactgctactgcaagcggtgctgcctgcactgccaggtgtgcttcaccaagaagggcctgggcatctcctacggccggaagaagcggaggcagaggcggagagccccccaggactccaagacccaccaggtgagcctgagcaagcagcccgcctcccagccccggggcgaccccaccggccccaaggagagcaagaagaaggtggagcgggagaccgagaccgaccctgaggactga

SEQ ID NO: 211 - RNA, 67 nt, synthetic construct
  source 1..67: mol_type = other RNA
agacccaagctacatttgcttctgacacaactgtgttcactagcaacctcaaacagacaccgccacc

SEQ ID NO: 212 - RNA, 38 nt, synthetic construct
  source 1..38: mol_type = other RNA
aaatagcccagaaattctacccaagctccctcgccacc

SEQ ID NO: 213 - RNA, 81 nt, synthetic construct
  source 1..81: mol_type = other RNA
aaatagctctctgctcctcctgttcgacagtcagccgcatcttcttttgcgtcgccagccgagccacatcgctcagccacc

SEQ ID NO: 214 - RNA, 88 nt, synthetic construct
  source 1..88: mol_type = other RNA
aaatacacatccgccgtcgtcgccgccatcctcggcgcgactcgcttctttcggttctacctgggagaatccaccgccatccgccacc

SEQ ID NO: 215 - RNA, 39 nt, synthetic construct
  source 1..39: mol_type = other RNA
aaatagtacctggtttttgttgtcagctggttagccacc

SEQ ID NO: 216 - RNA, 54 nt, synthetic construct
  source 1..54: mol_type = other RNA
aaatacatttgcttctgacacaactgtgttcactagcaacctcaaacagccacc

SEQ ID NO: 217 - RNA, 86 nt, synthetic construct
  source 1..86: mol_type = other RNA
aaatagttcagtcgggtcccggcagcggctgcagcgctctcgtcttctgcggctctcggtgccctctccttttcgtttccgccacc

SEQ ID NO: 218 - RNA, 63 nt, synthetic construct
  source 1..63: mol_type = other RNA
aaatacacttgctttgacacaactgtgtttacttgcaatcccccaaaacagacagacgccacc